European Patent Specification EP 3 706 801 B1, published January 14, 2026. Title: Platinum complexes and uses thereof. Applicant: L.E.A.F. HOLDINGS GROUP LLC NIYIKIZA, Clet MOYO, Victor M. Application to be assigned. The sequence listing filed with the application follows.

SEQUENCE LISTING (44 sequences)

SEQ ID NO: 1 - protein, 25 aa, Artificial Sequence
  synthetic construct
RQIKIWFQNRRMKWKKRKKRRQRRR

SEQ ID NO: 2 - protein, 11 aa, Artificial Sequence
  synthetic construct
  MISC_FEATURE (6)..(6): Xaa can be any naturally occurring amino acid
RKKRRXRRRGC

SEQ ID NO: 3 - DNA, 13 bp, Artificial Sequence
  synthetic construct
ccgccaagaagcg

SEQ ID NO: 4 - DNA, 100 bp, Artificial Sequence
  synthetic construct
gcgtgcacacgcgcgtagacttcccccgcaagtcactcgttagcccgccaagaagcgacccctccggggcgagctgagcggcgtggcgcgggggcgtcat

SEQ ID NO: 5 - DNA, 101 bp, Artificial Sequence
  synthetic construct
acgtgcatacgcacgtagacattccccgcttcccactccaaagtccgccaagaagcgtatcccgctgagcggcgtggcgcgggggcgtcatccgtcagctc

SEQ ID NO: 6 - DNA, 58 bp, Artificial Sequence
  synthetic construct
acttcccccgcaagtcactcgttagcccgccaagaagcgacccctccggggcgagctg

SEQ ID NO: 7 - protein, 9 aa, Artificial Sequence
  synthetic construct
RKKRRQRRR

SEQ ID NO: 8 - protein, 13 aa, Artificial Sequence
  synthetic construct
GRKKRRQRRRTPQ

SEQ ID NO: 9 - protein, 11 aa, Artificial Sequence
  synthetic construct
YGRKKRRQRRR

SEQ ID NO: 10 - protein, 15 aa, Artificial Sequence
  synthetic construct
AAVALLPAVLLALLA

SEQ ID NO: 11 - protein, 15 aa, Artificial Sequence
  synthetic construct
MGLGLHLLVLAAALQ

SEQ ID NO: 12 - protein, 15 aa, Artificial Sequence
  synthetic construct
GALFLGFLGAAGSTM

SEQ ID NO: 13 - protein, 21 aa, Artificial Sequence
  synthetic construct
AGYLLGKINLKALAALAKKIL

SEQ ID NO: 14 - protein, 16 aa, Artificial Sequence
  synthetic construct
RVIRVWFQNKRCKDKK

SEQ ID NO: 15 - protein, 16 aa, Artificial Sequence
  synthetic construct
RQIKIWFQNRRMKWKK

SEQ ID NO: 16 - protein, 20 aa, Artificial Sequence
  synthetic construct
GLFEAIAGFIENGWEGMIDG

SEQ ID NO: 17 - protein, 15 aa, Artificial Sequence
  synthetic construct
GWTLNSAGYLLGKIN

SEQ ID NO: 18 - protein, 15 aa, Artificial Sequence
  synthetic construct
RSQSRSRYYRQRQRS

SEQ ID NO: 19 - protein, 8 aa, Artificial Sequence
  synthetic construct
LAIPEQEY

SEQ ID NO: 20 - protein, 8 aa, Artificial Sequence
  synthetic construct
LGIAEQEY

SEQ ID NO: 21 - protein, 8 aa, Artificial Sequence
  synthetic construct
LGIPAQEY

SEQ ID NO: 22 - protein, 8 aa, Artificial Sequence
  synthetic construct
LGIPEAEY

SEQ ID NO: 23 - protein, 8 aa, Artificial Sequence
  synthetic construct
LGIPEQAY

SEQ ID NO: 24 - protein, 8 aa, Artificial Sequence
  synthetic construct
LGIAEAEY

SEQ ID NO: 25 - protein, 8 aa, Artificial Sequence
  synthetic construct
LGIPEAAY

SEQ ID NO: 26 - protein, 8 aa, Artificial Sequence
  synthetic construct
LGIAEQAY

SEQ ID NO: 27 - protein, 8 aa, Artificial Sequence
  synthetic construct
LGIAEAAY

SEQ ID NO: 28 - protein, 18 aa, Artificial Sequence
  synthetic construct
LLIILRRRIRKQAHAHSK

SEQ ID NO: 29 - protein, 12 aa, Artificial Sequence
  synthetic construct
LKALAALAKKIL

SEQ ID NO: 30 - protein, 18 aa, Artificial Sequence
  synthetic construct
KLALKLALKALKAALKLA

SEQ ID NO: 31 - protein, 21 aa, Artificial Sequence
  synthetic construct
KETWWETWWTEWSQPKKKRKV

SEQ ID NO: 32 - protein, 8 aa, Artificial Sequence
  synthetic construct
DHQLNPAF

SEQ ID NO: 33 - protein, 8 aa, Artificial Sequence
  synthetic construct
DPKGDPKG

SEQ ID NO: 34 - protein, 18 aa, Artificial Sequence
  synthetic construct
VTVTVTVTVTGKGDPKPD

SEQ ID NO: 35 - protein, 16 aa, Artificial Sequence
  synthetic construct
RQIKIWFQNRRMKWKK

SEQ ID NO: 36 - protein, 13 aa, Artificial Sequence
  synthetic construct
GRKKRRQRRRPPQ

SEQ ID NO: 37 - protein, 27 aa, Artificial Sequence
  synthetic construct
GWTLNSAGYLLGKINLKALAALAKKIL

SEQ ID NO: 38 - protein, 10 aa, Artificial Sequence
  synthetic construct
GRKKRRQRRR

SEQ ID NO: 39 - protein, 7 aa, Artificial Sequence
  synthetic construct
RRRRRRR

SEQ ID NO: 40 - protein, 8 aa, Artificial Sequence
  synthetic construct
RRRRRRRR

SEQ ID NO: 41 - protein, 9 aa, Artificial Sequence
  synthetic construct
RRRRRRRRR

SEQ ID NO: 42 - protein, 10 aa, Artificial Sequence
  synthetic construct
RRRRRRRRRR

SEQ ID NO: 43 - protein, 10 aa, Artificial Sequence
  synthetic construct
RRRRRRRRRR

SEQ ID NO: 44 - protein, 33 aa, Artificial Sequence
  synthetic construct
  MISC_FEATURE (33)..(33): Xaa can be 2 to 15 Arg independently in the L and/or D form
YTIWMPENPRPGTPCDIFTNSRGKRASNGGGGX